European Patent Specification EP 3 502 267 B1, published October 29, 2025. Title: METHODS AND COMPOSITIONS FOR PREVENTING NORLEUCINE MISINCORPORATION INTO PROTEINS. Applicant: GENENTECH, INC. ET AL. The sequence listing filed with the application follows.

SEQUENCE LISTING (52 sequences)

SEQ ID NO: 1 - DNA, 34 bp, Artificial Sequence
  source: /note="Description of Artificial Sequence: Synthetic primer"
cacacgagctcctcattttgctcattaacgttgg

SEQ ID NO: 2 - DNA, 25 bp, Artificial Sequence
  source: /note="Description of Artificial Sequence: Synthetic primer"
cacacgtcgacgcgaatggaagctg

SEQ ID NO: 3 - DNA, 30 bp, Artificial Sequence
  source: /note="Description of Artificial Sequence: Synthetic primer"
cacacgagctcgtatgcaaagcagagatgc

SEQ ID NO: 4 - DNA, 28 bp, Artificial Sequence
  source: /note="Description of Artificial Sequence: Synthetic primer"
cacacgtcgaccgtcattgccttgtttg

SEQ ID NO: 5 - DNA, 30 bp, Artificial Sequence
  source: /note="Description of Artificial Sequence: Synthetic primer"
gttctgatccttaacctgatgccgaagaag

SEQ ID NO: 6 - DNA, 24 bp, Artificial Sequence
  source: /note="Description of Artificial Sequence: Synthetic primer"
ccagcgtttgcgcatcatattcgg

SEQ ID NO: 7 - DNA, 28 bp, Artificial Sequence
  source: /note="Description of Artificial Sequence: Synthetic primer"
ggcaaaacacctttttacgtccgagtcc

SEQ ID NO: 8 - DNA, 27 bp, Artificial Sequence
  source: /note="Description of Artificial Sequence: Synthetic primer"
gaactcacgtaccagcagggtcagttg

SEQ ID NO: 9 - DNA, 26 bp, Artificial Sequence
  source: /note="Description of Artificial Sequence: Synthetic primer"
ccagtcacgacgttgtaaaacgacgg

SEQ ID NO: 10 - DNA, 25 bp, Artificial Sequence
  source: /note="Description of Artificial Sequence: Synthetic primer"
agtgaacggcaggtatatgtgatgg

SEQ ID NO: 11 - DNA, 31 bp, Artificial Sequence
  source: /note="Description of Artificial Sequence: Synthetic primer"
gtgatgacaacttcttgtgcgtctggtcagg

SEQ ID NO: 12 - DNA, 31 bp, Artificial Sequence
  source: /note="Description of Artificial Sequence: Synthetic primer"
cctgaccagacgcacaagaagttgtcatcac

SEQ ID NO: 13 - DNA, 30 bp, Artificial Sequence
  source: /note="Description of Artificial Sequence: Synthetic primer"
caaactcacctttggaggtcgatattcagc

SEQ ID NO: 14 - DNA, 30 bp, Artificial Sequence
  source: /note="Description of Artificial Sequence: Synthetic primer"
gctgaatatcgacctccaaaggtgagtttg

SEQ ID NO: 15 - DNA, 35 bp, Artificial Sequence
  source: /note="Description of Artificial Sequence: Synthetic primer"
gctcaactattacgtctgccagatcacgccatacg

SEQ ID NO: 16 - DNA, 35 bp, Artificial Sequence
  source: /note="Description of Artificial Sequence: Synthetic primer"
cgtatggcgtgatctggcagacgtaatagttgagc

SEQ ID NO: 17 - DNA, 30 bp, Artificial Sequence
  source: /note="Description of Artificial Sequence: Synthetic primer"
cgtctaccagagcacgctatacgatctacg

SEQ ID NO: 18 - DNA, 30 bp, Artificial Sequence
  source: /note="Description of Artificial Sequence: Synthetic primer"
cgtagatcgtatagcgtgctctggtagacg

SEQ ID NO: 19 - DNA, 27 bp, Artificial Sequence
  source: /note="Description of Artificial Sequence: Synthetic primer"
atcgatgctgtcgagctttccactcag

SEQ ID NO: 20 - DNA, 27 bp, Artificial Sequence
  source: /note="Description of Artificial Sequence: Synthetic primer"
ctgagtggaaagctcgacagcatcgat

SEQ ID NO: 21 - DNA, 24 bp, Artificial Sequence
  source: /note="Description of Artificial Sequence: Synthetic primer"
gcgcagctgctggcgatgctgccg

SEQ ID NO: 22 - DNA, 24 bp, Artificial Sequence
  source: /note="Description of Artificial Sequence: Synthetic primer"
cggcagcatcgccagcagctgcgc

SEQ ID NO: 23 - DNA, 930 bp, Artificial Sequence
  source: /note="Description of Artificial Sequence: Synthetic polynucleotide"
atgccgattcgtgtgccggacgagctacccgccgtcaatttcttgcgtgaagaaaacgtctttgtgatgacaacttcttgtgcgtctggtcaggaaattcgtccacttaaggttctgatccttaacctgatgccgaagaagattgaaactgaaaatcagtttctgcgcctgctttcaaactcacctttgcaggtcgatattcagctgttgcgcatcgattcccgtgaatcgcgcaacacgcccgcagagcatctgaacaacttctactgtaactttgaagatattcaggatcagaactttgacggtttgattgtaactggtgcgccgctgggcctggtggagtttaatgatgtcgcttactggccgcagatcaaacaggtgctggagtggtcgaaagatcacgtcacctcgacgctgtttgtctgctgggcggtacaggccgcgctcaatatcctctacggcattcctaagcaaactcgcaccgaaaaactctctggcgtttacgagcatcatattctccatcctcatgcgcttctgacgcgtggctttgatgattcattcctggcaccgcattcgcgctatgctgactttccggcagcgttgattcgtgattacaccgatctggaaattctggcagagacggaagaaggggatgcatatctgtttgccagtaaagataagcgcattgcctttgtgacgggccatcccgaatatgatgcgcaaacgctggcgcaggaatttttccgcgatgtggaagccggactagacccggatgtaccgtataactatttcccgcacaatgatccgcaaaatacaccgcgagcgagctggcgtagtcacggtaatttactgtttaccaactggctcaactattacgtctaccagatcacgccatacgatctacggcacatgaatccaacgctggattaa

SEQ ID NO: 24 - DNA, 930 bp, Artificial Sequence
  source: /note="Description of Artificial Sequence: Synthetic polynucleotide"
atgccgattcgtgtgccggacgagctacccgccgtcaatttcttgcgtgaagaaaacgtctttgtgatgacaacttctcgtgcgtctggtcaggaaattcgtccacttaaggttctgatccttaacctgatgccgaagaagattgaaactgaaaatcagtttctgcgcctgctttcaaactcacctttgcaggtcgatattcagctgttgcgcatcgattcccgtgaatcgcgcaacacgcccgcagagcatctgaacaacttctactgtaactttgaagatattcaggatcagaactttgacggtttgattgtaactggtgcgccgctgggcctggtggagtttaatgatgtcgcttactggccgcagatcaaacaggtgctggagtggtcgaaagatcacgtcacctcgacgctgtttgtctgctgggcggtacaggccgcgctcaatatcctctacggcattcctaagcaaactcgcaccgaaaaactctctggcgtttacgagcatcatattctccatcctcatgcgcttctgacgcgtggctttgatgattcattcctggcaccgcattcgcgctatgctgactttccggcagcgttgattcgtgattacaccgatctggaaattctggcagagacggaagaaggggatgcatatctgtttgccagtaaagataagcgcattgcctttgtgacgggccatcccgaatatgatgcgcaaacgctggcgcaggaatttttccgcgatgtggaagccggactagacccggatgtaccgtataactatttcccgcacaatgatccgcaaaatacaccgcgagcgagctggcgtagtcacggtaatttactgtttaccaactggctcaactattacgtctgccagatcacgccatacgatctacggcacatgaatccaacgctggattaa

SEQ ID NO: 25 - DNA, 930 bp, Artificial Sequence
  source: /note="Description of Artificial Sequence: Synthetic polynucleotide"
atgccgattcgtgtgccggacgagctacccgccgtcaatttcttgcgtgaagaaaacgtctttgtgatgacaacttctcgtgcgtctggtcaggaaattcgtccacttaaggttctgatccttaacctgatgccgaagaagattgaaactgaaaatcagtttctgcgcctgctttcaaactcacctttgcaggtcgatattcagctgttgcgcatcgattcccgtgaatcgcgcaacacgcccgcagagcatctgaacaacttctactgtaactttgaagatattcaggatcagaactttgacggtttgattgtaactggtgcgccgctgggcctggtggagtttaatgatgtcgcttactggccgcagatcaaacaggtgctggagtggtcgaaagatcacgtcacctcgacgctgtttgtctgctgggcggtacaggccgcgctcaatatcctctacggcattcctaagcaaactcgcaccgaaaaactctctggcgtttacgagcatcatattctccatcctcatgcgcttctgacgcgtggctttgatgattcattcctggcaccgcattcgcgctatgctgactttccggcagcgttgattcgtgattacaccgatctggaaattctggcagagacggaagaaggggatgcatatctgtttgccagtaaagataagcgcattgcctttgtgacgggccatcccgaatatgatgcgcaaacgctggcgcaggaatttttccgcgatgtggaagccggactagacccggatgtaccgtataactatttcccgcacaatgatccgcaaaatacaccgcgagcgagctggcgtagtcacggtaatttactgtttaccaactggctcaactattacgtctaccagagcacgctatacgatctacggcacatgaatccaacgctggattaa

SEQ ID NO: 26 - DNA, 930 bp, Artificial Sequence
  source: /note="Description of Artificial Sequence: Synthetic polynucleotide"
atgccgattcgtgtgccggacgagctacccgccgtcaatttcttgcgtgaagaaaacgtctttgtgatgacaacttctcgtgcgtctggtcaggaaattcgtccacttaaggttctgatccttaacctgatgccgaagaagattgaaactgaaaatcagtttctgcgcctgctttcaaactcacctttggaggtcgatattcagctgttgcgcatcgattcccgtgaatcgcgcaacacgcccgcagagcatctgaacaacttctactgtaactttgaagatattcaggatcagaactttgacggtttgattgtaactggtgcgccgctgggcctggtggagtttaatgatgtcgcttactggccgcagatcaaacaggtgctggagtggtcgaaagatcacgtcacctcgacgctgtttgtctgctgggcggtacaggccgcgctcaatatcctctacggcattcctaagcaaactcgcaccgaaaaactctctggcgtttacgagcatcatattctccatcctcatgcgcttctgacgcgtggctttgatgattcattcctggcaccgcattcgcgctatgctgactttccggcagcgttgattcgtgattacaccgatctggaaattctggcagagacggaagaaggggatgcatatctgtttgccagtaaagataagcgcattgcctttgtgacgggccatcccgaatatgatgcgcaaacgctggcgcaggaatttttccgcgatgtggaagccggactagacccggatgtaccgtataactatttcccgcacaatgatccgcaaaatacaccgcgagcgagctggcgtagtcacggtaatttactgtttaccaactggctcaactattacgtctaccagatcacgccatacgatctacggcacatgaatccaacgctggattaa

SEQ ID NO: 27 - DNA, 1155 bp, Artificial Sequence
  source: /note="Description of Artificial Sequence: Synthetic polynucleotide"
atggcaaaacacctttttacgtccgagtccgtctctgaagggcatcctgacaaaattgctgaccaaatttctgatgccgttttagacgcgatcctcgaacaggatccgaaagcacgcgttgcttgcgaaacctacgtaaaaaccggcatggttttagttggcggcgaaatcaccaccagcgcctgggtagacatcgaagagatcacccgtaacaccgttcgcgaaattggctatgtgcattccgacatgggctttgacgctaactcctgtgcggttctgagcgctatcggcaaacagtctcctgacatcaaccagggcgttgaccgtgccgatccgctggaacagggcgcgggtgaccagggtctgatgtttggctacgcaactaatgaaaccgacgtgctgatgccagcacctatcacctatgcacaccgtctggtacagcgtcaggctgaagtgcgtaaaaacggcactctgccgtggctgcgcccggacgcgaaaagccaggtgacttttcagtatgacgacggcaaaatcgttggtatcgatgctgtcgagctttccactcagcactctgaagagatcgaccagaaatcgctgcaagaagcggtaatggaagagatcatcaagccaattctgcccgctgaatggctgacttctgccaccaaattcttcatcaacccgaccggtcgtttcgttatcggtggcccaatgggtgactgcggtctgactggtcgtaaaattatcgttgatacctacggcggcatggcgcgtcacggtggcggtgcattctctggtaaagatccatcaaaagtggaccgttccgcagcctacgcagcacgttatgtcgcgaaaaacatcgttgctgctggcctggccgatcgttgtgaaattcaggtttcctacgcaatcggcgtggctgaaccgacctccatcatggtagaaactttcggtactgagaaagtgccttctgaacaactgaccctgctggtacgtgagttcttcgacctgcgcccatacggtctgattcagatgctggatctgctgcacccgatctacaaagaaaccgcagcatacggtcactttggtcgtgaacatttcccgtgggaaaaaaccgacaaagcgcagctgctgcgcgatgctgccggtctgaagtaa

SEQ ID NO: 28 - DNA, 1154 bp, Artificial Sequence
  source: /note="Description of Artificial Sequence: Synthetic polynucleotide"
atggcaaaacacctttttacgtccgagtccgtctctgaagggcatcctgacaaaattgctgaccaaatttctgatgccgttttagacgcgatcctcgaacaggatccgaaagcacgcgttgcttgcgaaacctacgtaaaaaccggcatggttttagttggcggcgaaatcaccaccagcgcctgggtagacatcgaagagatcacccgtaacaccgttcgcgaaattggctatgtgcattccgacatgggctttgacgctaactcctgtgcggttctgagcgctatcggcaaacagtctcctgacatcaaccagggcgttgaccgtgccgatccgctggaacagggcgcgggtgaccagggtctgatgtttggctacgcaactaatgaaaccgacgtgctgatgccagcacctatcacctatgcacaccgtctggtacagcgtcaggctgaagtgcgtaaaaacggcactctgccgtggctgcgcccggacgcgaaaagccaggtgacttttcagtatgacgacggcaaaatcgttggtatcgatgctgtcgtgctttccactcagcactctgaagagatcgaccagaaatcgctgcaagaagcggtaatggaagagatcatcaagccaattctgcccgctgaatggctgacttctgccaccaaattcttcatcaacccgaccggtcgtttcgttatcggtggcccaatgggtgactgcggtctgactggtcgtaaaattatcgttgatacctacggcggcatggcgcgtcacggtggcggtgcattctctggtaaagatccatcaaaagtggaccgttccgcagcctacgcagcacgttatgtcgcgaaaaacatcgttgctgctggcctggccgatcgttgtgaaattcaggtttcctacgcaatcggcgtggctgaaccgacctccatcatggtagaaactttcggtactgagaaagtgccttctgaacaactgaccctgctggtacgtgagttcttcgacctgcgcccatacggtctgattcagatgctggatctgctgcacccgatctacaaagaaaccgcagcatacggtcactttggtcgtgaacatttcccgtgggaaaaaaccgacaaagcgcagctgctggcgatgctgccggtctgaagtaa

SEQ ID NO: 29 - protein, 308 aa, Escherichia coli
MPIRVPDELPAVNFLREENVFVMTTSRASGQEIRPLKVLILNLMPKKIETENQFLRLLSNSPLQVDIQLLRIDSRESRNTPAEHLNNFYCNFEDIQDQNFDGLIVTGAPLGLVEFNDVAYWPQIKQVLEWSKDHVTSTLFVCWAVQAALNILYGIPKQTRTEKLSGVYEHHILHPHALLTRGFDDSFLAHSRYADFPAALIRDYTDLEILAETEEGDAYLFASKDKRIAFVTGHPEYDAQTLAQEFFRDVEAGLDPDVPYNYFPHNDPQNTPRASWRSHGNLLFTNWLNYYVYQITPYDLRHMNPTLD

SEQ ID NO: 30 - protein, 384 aa, Escherichia coli
MAKHLFTSESVSEGHPDKIADQISDAVLDAILEQDPKARVACETYVKTGMVLVGGEITTSAWVDIEEITRNTVREIGYVHSDMGFDANSCAVLSAIGKQSPDINQGVDRADPLEQGAGDQGLMFGYATNETDVLMPAPITYAHRLVQRQAEVRKNGTLPWLRPDAKSQVTFQYDDGKIVGIDAVVLSTQHSEEIDQKSLQEAVMEEIIKPILPAEWLTSATKFFINPTGRFVIGGPMGDCGLTGRKIIVDTYGGMARHGGGAFSGKDPSKVDRSAAYAARYVAKNIVAAGLADRCEIQVSYAIGVAEPTSIMVETFGTEKVPSEQLTLLVREFFDLRPYGLIQMLDLLHPIYKETAAYGHFGREHFPWEKTDKAQLLRDAAGLK

SEQ ID NO: 31 - DNA, 930 bp, Escherichia coli; identical to SEQ ID NO: 23

SEQ ID NO: 32 - DNA, 1155 bp, Escherichia coli
atggcaaaacacctttttacgtccgagtccgtctctgaagggcatcctgacaaaattgctgaccaaatttctgatgccgttttagacgcgatcctcgaacaggatccgaaagcacgcgttgcttgcgaaacctacgtaaaaaccggcatggttttagttggcggcgaaatcaccaccagcgcctgggtagacatcgaagagatcacccgtaacaccgttcgcgaaattggctatgtgcattccgacatgggctttgacgctaactcctgtgcggttctgagcgctatcggcaaacagtctcctgacatcaaccagggcgttgaccgtgccgatccgctggaacagggcgcgggtgaccagggtctgatgtttggctacgcaactaatgaaaccgacgtgctgatgccagcacctatcacctatgcacaccgtctggtacagcgtcaggctgaagtgcgtaaaaacggcactctgccgtggctgcgcccggacgcgaaaagccaggtgacttttcagtatgacgacggcaaaatcgttggtatcgatgctgtcgtgctttccactcagcactctgaagagatcgaccagaaatcgctgcaagaagcggtaatggaagagatcatcaagccaattctgcccgctgaatggctgacttctgccaccaaattcttcatcaacccgaccggtcgtttcgttatcggtggcccaatgggtgactgcggtctgactggtcgtaaaattatcgttgatacctacggcggcatggcgcgtcacggtggcggtgcattctctggtaaagatccatcaaaagtggaccgttccgcagcctacgcagcacgttatgtcgcgaaaaacatcgttgctgctggcctggccgatcgttgtgaaattcaggtttcctacgcaatcggcgtggctgaaccgacctccatcatggtagaaactttcggtactgagaaagtgccttctgaacaactgaccctgctggtacgtgagttcttcgacctgcgcccatacggtctgattcagatgctggatctgctgcacccgatctacaaagaaaccgcagcatacggtcactttggtcgtgaacatttcccgtgggaaaaaaccgacaaagcgcagctgctgcgcgatgctgccggtctgaagtaa

SEQ ID NO: 33 - DNA, 642 bp, Artificial Sequence
  source: /note="Description of Artificial Sequence: Synthetic polynucleotide"
gatatccagttgacccagtccccgagctccctgtccgcctctgtgggcgatagggtcaccatcacctgcagcgcaagtcaggatattagcaactatttaaactggtatcaacagaaaccaggaaaagctccgaaagtactgatttacttcacctcctctctccactctggagtcccttctcgcttctctggatccggttctgggacggatttcactctgaccatcagcagtctgcagccagaagacttcgcaacttattactgtcaacagtatagcaccgtgccgtggacgtttggacagggtaccaaggtggagatcaaacgaactgtggctgcaccatctgtcttcatcttcccgccatctgatgagcagttgaaatctggaactgcttctgttgtgtgcctgctgaataacttctatcccagagaggccaaagtacagtggaaggtggataacgccctccaatcgggtaactcccaggagagtgtcacagagcaggacagcaaggacagcacctacagcctcagcagcaccctgacgctgagcaaagcagactacgagaaacacaaagtctacgcctgcgaagtcacccatcagggcctgagctcgcccgtcacaaagagcttcaacaggggagagtgt

SEQ ID NO: 34 - DNA, 693 bp, Artificial Sequence
  source: /note="Description of Artificial Sequence: Synthetic polynucleotide"
gaggttcagctggtggagtctggcggtggcctggtgcagccagggggctcactccgtttgtcctgtgcagcttctggctacgacttcacgcactacggtatgaactgggtccgtcaggccccgggtaagggcctggaatgggttggatggattaacacctataccggtgaaccgacctatgctgcggatttcaaacgtcgtttcactttttctttagacacctccaaaagcacagcatacctgcagatgaacagcctgcgcgctgaggacactgccgtctattactgtgcaaagtacccgtactattatgggacgagccactggtatttcgacgtctggggtcaaggaaccctggtcaccgtctcctcggcctccaccaagggcccatcggtcttccccctggcaccctcctccaagagcacctctgggggcacagcggccctgggctgcctggtcaaggactacttccccgaaccggtgacggtgtcgtggaactcaggcgccctgaccagcggcgtgcacaccttcccggctgtcctacagtcctcaggactctactccctcagcagcgtggtgaccgtgccctccagcagcttgggcacccagacctacatctgcaacgtgaatcacaagcccagcaacaccaaggtcgacaagaaagttgagcccaaatcttgtgacaaaactcacctc

SEQ ID NO: 35 - protein, 19 aa, Artificial Sequence
  source: /note="Description of Artificial Sequence: Synthetic peptide"
LSCAASGYDFTHYGMNWVR

SEQ ID NO: 36 - protein, 11 aa, Artificial Sequence
  source: /note="Description of Artificial Sequence: Synthetic peptide"
STAYLQMNSLR

SEQ ID NO: 37 - protein, 15 aa, Artificial Sequence
  source: /note="Description of Artificial Sequence: Synthetic peptide"
ASGYTFTNYGMNWVR

SEQ ID NO: 38 - protein, 27 aa, Artificial Sequence
  source: /note="Description of Artificial Sequence: Synthetic peptide"
QAPGQGLEWMGWINTYTGETTYADDFK

SEQ ID NO: 39 - protein, 24 aa, Artificial Sequence
  source: /note="Description of Artificial Sequence: Synthetic peptide"
VTITCITSTDIDDDMNWYQQKPGK

SEQ ID NO: 40 - protein, 16 aa, Artificial Sequence
  source: /note="Description of Artificial Sequence: Synthetic peptide"
GLEWVGMIDPSNSDTR

SEQ ID NO: 41 - protein, 11 aa, Artificial Sequence
  source: /note="Description of Artificial Sequence: Synthetic peptide"
NTAYLQMNSLR

SEQ ID NO: 42 - protein, 7 aa, Artificial Sequence
  source: /note="Description of Artificial Sequence: Synthetic peptide"
DTLMISR

SEQ ID NO: 43 - protein, 5 aa, Artificial Sequence
  source: /note="Description of Artificial Sequence: Synthetic peptide"
EEMTK

SEQ ID NO: 44 - protein, 23 aa, Artificial Sequence
  source: /note="Description of Artificial Sequence: Synthetic peptide"
WQQGNVFSCSVMHEALHNHYTQK

SEQ ID NO: 45 - protein, 18 aa, Artificial Sequence
  source: /note="Description of Artificial Sequence: Synthetic peptide"
DIQMTQSPSSLSASVGDR

SEQ ID NO: 46 - protein, 214 aa, Artificial Sequence
  source: /note="Description of Artificial Sequence: Synthetic polypeptide"
DIQLTQSPSSLSASVGDRVTITCSASQDISNYLNWYQQKPGKAPKVLIYFTSSLHSGVPSRFSGSGSGTDFTLTISSLQPEDFATYYCQQYSTVPWTFGQGTKVEIKRTVAAPSVFIFPPSDEQLKSGTASVVCLLNNFYPREAKVQWKVDNALQSGNSQESVTEQDSKDSTYSLSSTLTLSKADYEKHKVYACEVTHQGLSSPVTKSFNRGEC

SEQ ID NO: 47 - protein, 231 aa, Artificial Sequence
  source: /note="Description of Artificial Sequence: Synthetic polypeptide"
EVQLVESGGGLVQPGGSLRLSCAASGYDFTHYGMNWVRQAPGKGLEWVGWINTYTGEPTYAADFKRRFTFSLDTSKSTAYLQMNSLRAEDTAVYYCAKYPYYYGTSHWYFDVWGQGTLVTVSSASTKGPSVFPLAPSSKSTSGGTAALGCLVKDYFPEPVTVSWNSGALTSGVHTFPAVLQSSGLYSLSSVVTVPSSSLGTQTYICNVNHKPSNTKVDKKVEPKSCDKTHL

SEQ ID NO: 48 - protein, 214 aa, Artificial Sequence
  source: /note="Description of Artificial Sequence: Synthetic polypeptide"
DIQVTQSPSSLSASVGDRVTITCITSTDIDDDMNWYQQKPGKVPKLLISGGNTLRPGVPSRFSGSGSGTDFTLTISSLQPEDVATYYCLQSDSLPYTFGQGTKVEIKRTVAAPSVFIFPPSDEQLKSGTASVVCLLNNFYPREAKVQWKVDNALQSGNSQESVTEQDSKDSTYSLSSTLTLSKADYEKHKVYACEVTHQGLSSPVTKSFNRGEC

SEQ ID NO: 49 - protein, 223 aa, Artificial Sequence
  source: /note="Description of Artificial Sequence: Synthetic polypeptide"
EVQLVQSGPELKKPGASVKVSCKASGYTFTNYGMNWVRQAPGQGLEWMGWINTYTGETTYADDFKGRFVFSLDTSVSTAYLQISSLKAEDTAVYYCEREGGVNNWGQGTLVTVSSASTKGPSVFPLAPSSKSTSGGTAALGCLVKDYFPEPVTVSWNSGALTSGVHTFPAVLQSSGLYSLSSVVTVPSSSLGTQTYICNVNHKPSNTKVDKKVEPKSCDKTHT

SEQ ID NO: 50 - protein, 220 aa, Artificial Sequence
  source: /note="Description of Artificial Sequence: Synthetic polypeptide"
DIQMTQSPSSLSASVGDRVTITCKSSQSLLYTSSQKNYLAWYQQKPGKAPKLLIYWASTRESGVPSRFSGSGSGTDFTLTISSLQPEDFATYYCQQYYAYPWTFGQGTKVEIKRTVAAPSVFIFPPSDEQLKSGTASVVCLLNNFYPREAKVQWKVDNALQSGNSQESVTEQDSKDSTYSLSSTLTLSKADYEKHKVYACEVTHQGLSSPVTKSFNRGEC

SEQ ID NO: 51 - protein, 449 aa, Artificial Sequence
  source: /note="Description of Artificial Sequence: Synthetic polypeptide"
EVQLVESGGGLVQPGGSLRLSCAASGYTFTSYWLHWVRQAPGKGLEWVGMIDPSNSDTRFNPNFKDRFTISADTSKNTAYLQMNSLRAEDTAVYYCATYRSYVTPLDYWGQGTLVTVSSASTKGPSVFPLAPSSKSTSGGTAALGCLVKDYFPEPVTVSWNSGALTSGVHTFPAVLQSSGLYSLSSVVTVPSSSLGTQTYICNVNHKPSNTKVDKKVEPKSCDKTHTCPPCPAPELLGGPSVFLFPPKPKDTLMISRTPEVTCVVVDVSHEDPEVKFNWYVDGVEVHNAKTKPREEQYNSTYRVVSVLTVLHQDWLNGKEYKCKVSNKALPAPIEKTISKAKGQPREPQVYTLPPSREEMTKNQVSLSCAVKGFYPSDIAVEWESNGQPENNYKTTPPVLDSDGSFFLVSKLTVDKSRWQQGNVFSCSVMHEALHNHYTQKSLSLSPGK

SEQ ID NO: 52 - protein, 227 aa, Artificial Sequence
  source: /note="Description of Artificial Sequence: Synthetic polypeptide"
DKTHTCPPCPAPELLGGPSVFLFPPKPKDTLMISRTPEVTCVVVDVSHEDPEVKFNWYVDGVEVHNAKTKPREEQYNSTYRVVSVLTVLHQDWLNGKEYKCKVSNKALPAPIEKTISKAKGQPREPQVYTLPPSREEMTKNQVSLWCLVKGFYPSDIAVEWESNGQPENNYKTTPPVLDSDGSFFLYSKLTVDKSRWQQGNVFSCSVMHEALHNHYTQKSLSLSPGK